European Patent Specification EP 3 851 539 B1, published January 7, 2026. Title: METHODS AND PROCESSES FOR NON-INVASIVE ASSESSMENT OF CHROMOSOME ALTERATIONS. Applicant: SEQUENOM, INC. The sequence listing filed with the application follows.

SEQUENCE LISTING (4 sequences)

SEQ ID NO: 1 - DNA, 50 bp, Homo sapiens
cagattgagagtcgatccacagacagcctagcagagcaatccaagagtaa

SEQ ID NO: 2 - DNA, 50 bp, Homo sapiens
cagattgagagtcgatccacagacaagggcggggctgggttttagccgta

SEQ ID NO: 3 - DNA, 50 bp, Homo sapiens
acaactggaggatctgggcgcctcgagggcggggctgggttttagccgta

SEQ ID NO: 4 - DNA, 44 bp, Homo sapiens
acaactggaggatctgggcgcctagcagagcaatccaagagtaa